European Patent Specification EP 3 800 269 B1, published March 20, 2024. Title: Methods for detecting multiple nucleic acids in a sample. Applicant: Alere Technologies GmbH. The sequence listing filed with the application follows.

SEQUENCE LISTING (5 sequences)

SEQ ID NO: 1 - DNA, 33 bp, Artificial Sequence
  reverse primer Tb_DR_R25c
agactccatatggagtctcatctttccgtcccc

SEQ ID NO: 2 - DNA, 33 bp, Artificial Sequence
  forward primer Tb_DR_F16
cgactccatatggagtcgtcgtcagacccaaaa

SEQ ID NO: 3 - DNA, 23 bp, Artificial Sequence
  molecular beacon MB_P2_7
tcggggcagacccaaaaccccga

SEQ ID NO: 4 - DNA, 17 bp, Artificial Sequence
  reporter compound Anti_Tb_Target_CMA
cccaaaaccccgagagg

SEQ ID NO: 5 - DNA, 23 bp, Artificial Sequence
  reporter compound (positive hybridization control)
ccgactactacgggacgctggga